European Patent Application EP 4 729 129 A2, published April 22, 2026. Title: LIQUID COMPOSITION COMPRISING ANTIBODY OF HUMAN INTERLEUKIN-4 RECEPTOR ALPHA. Applicant: Connect Biopharma HongKong Limited. Application EP. The sequence listing filed with the application follows.

SEQUENCE LISTING (12 sequences)

SEQ ID NO: 1 - protein, 12 aa, synthetic construct
  REGION 1..12: note = Light chain variable region, CDR1
RASQSVSSSYLA

SEQ ID NO: 2 - protein, 7 aa, synthetic construct
  REGION 1..7: note = Light chain variable region, CDR2
GASSRAT

SEQ ID NO: 3 - protein, 10 aa, synthetic construct
  REGION 1..10: note = Light chain variable region, CDR3
QQYDHSAGWT

SEQ ID NO: 4 - protein, 109 aa, synthetic construct
  REGION 1..109: note = Light chain variable region
EIVLTQSPGTLSLSPGERATLSCRASQSVSSSYLAWYQQKPGQAPRLLIYGASSRATGIPDRFSGSGSGTDFTLTISRLEPEDFAVYYCQQYDHSAGWTFGQGTKVEIK

SEQ ID NO: 5 - protein, 5 aa, synthetic construct
  REGION 1..5: note = Heavy chain variable region, CDR1
RNAMF

SEQ ID NO: 6 - protein, 17 aa, synthetic construct
  REGION 1..17: note = Heavy chain variable region, CDR2
GIGTGGATSYADSVKGR

SEQ ID NO: 7 - protein, 7 aa, synthetic construct
  REGION 1..7: note = Heavy chain variable region, CDR3
GRYYFDY

SEQ ID NO: 8 - protein, 115 aa, synthetic construct
  REGION 1..115: note = Heavy chain variable region
EVQLVESGGGLVQPGGSLRLSCAASGFTFSRNAMFWVRQAPGKGLEWVSGIGTGGATSYADSVKGRFTISRDNAKNSLYLQMNSLRAEDTAVYYCARGRYYFDYWGQGTLVTVSS

SEQ ID NO: 9 - protein, 107 aa, synthetic construct [sequence omitted]

SEQ ID NO: 10 - protein, 326 aa, synthetic construct
  REGION 1..326: note = Heavy chain constant region
ASTKGPSVFPLAPCSRSTSESTAALGCLVKDYFPEPVTVSWNSGALTSGVHTFPAVLQSSGLYSLSSVVTVPSSSLGTKTYTCNVDHKPSNTKVDKRVESKYGPPCPPCPAPEFLGGPSVFLFPPKPKDTLMISRTPEVTCVVVDVSQEDPEVQFNWYVDGVEVHNAKTKPREEQFNSTYRVVSVLTVLHQDWLNGKEYKCKVSNKGLPSSIEKTISKAKGQPREPQVYTLPPSQEEMTKNQVSLTCLVKGFYPSDIAVEWESNGQPENNYKTTPPVLDSDGSFFLYSRLTVDKSRWQEGNVFSCSVMHEALHNHYTQKSLSLSLG

SEQ ID NO: 11 - protein, 216 aa, synthetic construct
  REGION 1..216: note = Light chain
EIVLTQSPGTLSLSPGERATLSCRASQSVSSSYLAWYQQKPGQAPRLLIYGASSRATGIPDRFSGSGSGTDFTLTISRLEPEDFAVYYCQQYDHSAGWTFGQGTKVEIKRTVAAPSVFIFPPSDEQLKSGTASVVCLLNNFYPREAKVQWKVDNALQSGNSQESVTEQDSKDSTYSLSSTLTLSKADYEKHKVYACEVTHQGLSSPVTKSFNRGEC

SEQ ID NO: 12 - protein, 441 aa, synthetic construct
  REGION 1..441: note = Heavy chain
EVQLVESGGGLVQPGGSLRLSCAASGFTFSRNAMFWVRQAPGKGLEWVSGIGTGGATSYADSVKGRFTISRDNAKNSLYLQMNSLRAEDTAVYYCARGRYYFDYWGQGTLVTVSSASTKGPSVFPLAPCSRSTSESTAALGCLVKDYFPEPVTVSWNSGALTSGVHTFPAVLQSSGLYSLSSVVTVPSSSLGTKTYTCNVDHKPSNTKVDKRVESKYGPPCPPCPAPEFLGGPSVFLFPPKPKDTLMISRTPEVTCVVVDVSQEDPEVQFNWYVDGVEVHNAKTKPREEQFNSTYRVVSVLTVLHQDWLNGKEYKCKVSNKGLPSSIEKTISKAKGQPREPQVYTLPPSQEEMTKNQVSLTCLVKGFYPSDIAVEWESNGQPENNYKTTPPVLDSDGSFFLYSRLTVDKSRWQEGNVFSCSVMHEALHNHYTQKSLSLSLG